European Patent Application EP 4 556 490 A1, published May 21, 2025. Title: Antibodies neutralizing SARS-CoV2. Applicant: SCRIPPS KOREA ANTIBODY INSTITUTE. The sequence listing filed with the application follows.

SEQUENCE LISTING (79 sequences)

SEQ ID NO: 1 - protein, 22 aa, synthetic construct
  REGION 1..22: note = L-FR1
QSVLTQPPSASGTPGRRVTISC

SEQ ID NO: 2 - protein, 15 aa, synthetic construct
  REGION 1..15: note = L-FR2
WYQQLPGTAPKLLIY

SEQ ID NO: 3 - protein, 35 aa, synthetic construct
  REGION 1..35: note = L-FR3
RPSGVPDRFSGSKSGTSASLAISGLRSEDEADYYC

SEQ ID NO: 4 - protein, 12 aa, synthetic construct
  REGION 1..12: note = L-FR4
YVFGGGTKLTVL

SEQ ID NO: 5 - protein, 30 aa, synthetic construct
  REGION 1..30: note = H-FR1
EVQLLESGGGLVQTGGSLRLSCAASGFTFS

SEQ ID NO: 6 - protein, 14 aa, synthetic construct
  REGION 1..14: note = H-FR2
WVRQAPGKGLEWVS

SEQ ID NO: 7 - protein, 39 aa, synthetic construct
  REGION 1..39: note = H-FR3
YYADSVKGRFTISRDNSKNTLYLQMNSLRAEDTAVYYCA

SEQ ID NO: 8 - protein, 9 aa, synthetic construct
  REGION 1..9: note = H-FR4
WGQGTLVTV

SEQ ID NO: 9 - protein, 13 aa, synthetic construct
  REGION 1..13: note = L-CDR1 (SKAI-DS1)
TGSSSNIGSNYVS

SEQ ID NO: 10 - protein, 13 aa, synthetic construct
  REGION 1..13: note = L-CDR1 (SKAI-DS3)
TGSSSNIGSNDVT

SEQ ID NO: 11 - protein, 13 aa, synthetic construct
  REGION 1..13: note = L-CDR1 (SKAI-DS7, SKAI-DS10, SKAI-DS17, SKAI-DS42, SKAI-DS64,SKAI-DS77)
SGSSSNIGSNAVS

SEQ ID NO: 12 - protein, 13 aa, synthetic construct
  REGION 1..13: note = L-CDR1 (SKAI-DS14)
SGSSSNIGSTNVY

SEQ ID NO: 13 - protein, 13 aa, synthetic construct
  REGION 1..13: note = L-CDR1 (SKAI-DS15)
SGSSSNIGSNDVN

SEQ ID NO: 14 - protein, 13 aa, synthetic construct
  REGION 1..13: note = L-CDR1 (SKAI-DS16)
SGSSSNIGSNYVY

SEQ ID NO: 15 - protein, 13 aa, synthetic construct
  REGION 1..13: note = L-CDR1 (SKAI-DS63)
SGSSSNIGSNTVS

SEQ ID NO: 16 - protein, 13 aa, synthetic construct
  REGION 1..13: note = L-CDR1 (SKAI-DS66)
TGSSSNIGSNAVY

SEQ ID NO: 17 - protein, 13 aa, synthetic construct
  REGION 1..13: note = L-CDR1 (SKAI-DS84)
TGSSSNIGNNSVT

SEQ ID NO: 18 - protein, 13 aa, synthetic construct
  REGION 1..13: note = L-CDR1 (SKAI-DS95)
TGSSSNIGSNSVT

SEQ ID NO: 19 - protein, 13 aa, synthetic construct
  REGION 1..13: note = L-CDR1 (SKAI-DS104)
TGSSSNIGNNTVN

SEQ ID NO: 20 - protein, 4 aa, synthetic construct
  REGION 1..4: note = L-CDR2 (SKAI-DS1)
SDSN

SEQ ID NO: 21 - protein, 4 aa, synthetic construct
  REGION 1..4: note = L-CDR2 (SKAI-DS3)
ADSK

SEQ ID NO: 22 - protein, 4 aa, synthetic construct
  REGION 1..4: note = L-CDR2 (SKAI-DS7, SKAI-DS10, SKAI-DS17, SKAI-DS42, SKAI-DS64,SKAI-DS77)
DNNH

SEQ ID NO: 23 - protein, 4 aa, synthetic construct
  REGION 1..4: note = L-CDR2 (SKAI-DS14, SKAI-DS104)
SDNK

SEQ ID NO: 24 - protein, 4 aa, synthetic construct
  REGION 1..4: note = L-CDR2 (SKAI-DS15, SKAI-DS16, SKAI-DS66)
DDSN

SEQ ID NO: 25 - protein, 4 aa, synthetic construct
  REGION 1..4: note = L-CDR2 (SKAI-DS63)
ADNN

SEQ ID NO: 26 - protein, 4 aa, synthetic construct
  REGION 1..4: note = L-CDR2 (SKAI-DS84)
ADSH

SEQ ID NO: 27 - protein, 4 aa, synthetic construct
  REGION 1..4: note = L-CDR2 (SKAI-DS95)
DDNQ

SEQ ID NO: 28 - protein, 9 aa, synthetic construct
  REGION 1..9: note = L-CDR3 (SKAI-DS1)
GTWDASLSG

SEQ ID NO: 29 - protein, 9 aa, synthetic construct
  REGION 1..9: note = L-CDR3 (SKAI-DS3)
GAWDYSLSA

SEQ ID NO: 30 - protein, 9 aa, synthetic construct
  REGION 1..9: note = L-CDR3 (SKAI-DS7, SKAI-DS10, SKAI-DS64, SKAI-DS77)
GSWDDSLNA

SEQ ID NO: 31 - protein, 9 aa, synthetic construct
  REGION 1..9: note = L-CDR3 (SKAI-DS14)
ASWDASLNG

SEQ ID NO: 32 - protein, 9 aa, synthetic construct
  REGION 1..9: note = L-CDR3 (SKAI-DS15)
GAWDDSLSG

SEQ ID NO: 33 - protein, 9 aa, synthetic construct
  REGION 1..9: note = L-CDR3 (SKAI-DS16)
GTWDYSLNG

SEQ ID NO: 34 - protein, 9 aa, synthetic construct
  REGION 1..9: note = L-CDR3 (SKAI-DS17)
GSWDDSLNA

SEQ ID NO: 35 - protein, 9 aa, synthetic construct
  REGION 1..9: note = L-CDR3 (SKAI-DS42)
GSWDDSLNG

SEQ ID NO: 36 - protein, 9 aa, synthetic construct
  REGION 1..9: note = L-CDR3 (SKAI-DS63)
AAWDDSLSA

SEQ ID NO: 37 - protein, 9 aa, synthetic construct
  REGION 1..9: note = L-CDR3 (SKAI-DS66)
GSWDDSLSA

SEQ ID NO: 38 - protein, 9 aa, synthetic construct
  REGION 1..9: note = L-CDR3 (SKAI-DS84)
GAWDDSLSG

SEQ ID NO: 39 - protein, 9 aa, synthetic construct
  REGION 1..9: note = L-CDR3 (SKAI-DS95)
AAWDDSLSG

SEQ ID NO: 40 - protein, 9 aa, synthetic construct
  REGION 1..9: note = L-CDR3 (SKAI-DS104)
AAWDASLSA

SEQ ID NO: 41 - protein, 5 aa, synthetic construct
  REGION 1..5: note = H-CDR1 (SKAI-DS1, SKAI-DS7, SKAI-DS10, SKAI-DS17, SKAI-DS66,SKAI-DS104)
DYAMS

SEQ ID NO: 42 - protein, 5 aa, synthetic construct
  REGION 1..5: note = H-CDR1 (SKAI-DS3, SKAI-DS16, SKAI-DS64)
DYSMS

SEQ ID NO: 43 - protein, 5 aa, synthetic construct
  REGION 1..5: note = H-CDR1 (SKAI-DS14, SKAI-DS15)
DYDMS

SEQ ID NO: 44 - protein, 5 aa, synthetic construct
  REGION 1..5: note = H-CDR1 (SKAI-DS42)
NYSMS

SEQ ID NO: 45 - protein, 5 aa, synthetic construct
  REGION 1..5: note = H-CDR1 (SKAI-DS63)
NYAMS

SEQ ID NO: 46 - protein, 5 aa, synthetic construct
  REGION 1..5: note = H-CDR1 (SKAI-DS77, SKAI-DS84)
DYYMS

SEQ ID NO: 47 - protein, 5 aa, synthetic construct
  REGION 1..5: note = H-CDR1 (SKAI-DS95)
GYDMS

SEQ ID NO: 48 - protein, 9 aa, synthetic construct
  REGION 1..9: note = H-CDR2 (SKAI-DS1)
WIYSNDGNK

SEQ ID NO: 49 - protein, 9 aa, synthetic construct
  REGION 1..9: note = H-CDR2 (SKAI-DS3)
AISSDSSST

SEQ ID NO: 50 - protein, 9 aa, synthetic construct
  REGION 1..9: note = H-CDR2 (SKAI-DS7)
GIYHSGGNT

SEQ ID NO: 51 - protein, 9 aa, synthetic construct
  REGION 1..9: note = H-CDR2 (SKAI-DS10)
EIYYHDSNT

SEQ ID NO: 52 - protein, 9 aa, synthetic construct
  REGION 1..9: note = H-CDR2 (SKAI-DS14)
VISYNGGSI

SEQ ID NO: 53 - protein, 9 aa, synthetic construct
  REGION 1..9: note = H-CDR2 (SKAI-DS15)
MIYSGSSSK

SEQ ID NO: 54 - protein, 9 aa, synthetic construct
  REGION 1..9: note = H-CDR2 (SKAI-DS16)
WIYPDNGNT

SEQ ID NO: 55 - protein, 9 aa, synthetic construct
  REGION 1..9: note = H-CDR2 (SKAI-DS17)
VIYYDGSSK

SEQ ID NO: 56 - protein, 9 aa, synthetic construct
  REGION 1..9: note = H-CDR2 (SKAI-DS42)
AISYDNGNK

SEQ ID NO: 57 - protein, 10 aa, synthetic construct
  REGION 1..10: note = H-CDR2 (SKAI-DS63)
GIYPNSGSNT

SEQ ID NO: 58 - protein, 9 aa, synthetic construct
  REGION 1..9: note = H-CDR2 (SKAI-DS64)
GIYHSDGSK

SEQ ID NO: 59 - protein, 9 aa, synthetic construct
  REGION 1..9: note = H-CDR2 (SKAI-DS66)
AIYPGGGST

SEQ ID NO: 60 - protein, 9 aa, synthetic construct
  REGION 1..9: note = H-CDR2 (SKAI-DS77)
AISYDDGNI

SEQ ID NO: 61 - protein, 9 aa, synthetic construct
  REGION 1..9: note = H-CDR2 (SKAI-DS84)
LISHGGSSK

SEQ ID NO: 62 - protein, 9 aa, synthetic construct
  REGION 1..9: note = H-CDR2 (SKAI-DS95)
GISYNNGST

SEQ ID NO: 63 - protein, 9 aa, synthetic construct
  REGION 1..9: note = H-CDR2 (SKAI-DS104)
WIYPDDGNT

SEQ ID NO: 64 - protein, 19 aa, synthetic construct
  REGION 1..19: note = H-CDR3 (SKAI-DS1)
RFPVPSWRNTWSSYDAMDV

SEQ ID NO: 65 - protein, 19 aa, synthetic construct
  REGION 1..19: note = H-CDR3 (SKAI-DS3)
KAILRCIPLGCYYADAMDV

SEQ ID NO: 66 - protein, 8 aa, synthetic construct
  REGION 1..8: note = H-CDR3 (SKAI-DS7)
RDAGPFDY

SEQ ID NO: 67 - protein, 8 aa, synthetic construct
  REGION 1..8: note = H-CDR3 (SKAI-DS10)
RGTGPFDY

SEQ ID NO: 68 - protein, 13 aa, synthetic construct
  REGION 1..13: note = H-CDR3 (SKAI-DS14)
KGVPEIAPPRFDY

SEQ ID NO: 69 - protein, 19 aa, synthetic construct
  REGION 1..19: note = H-CDR3 (SKAI-DS15)
RVTGTCHSGSCYYSDAMDV

SEQ ID NO: 70 - protein, 8 aa, synthetic construct
  REGION 1..8: note = H-CDR3 (SKAI-DS16)
KPKTSFDY

SEQ ID NO: 71 - protein, 8 aa, synthetic construct
  REGION 1..8: note = H-CDR3 (SKAI-DS17)
RDFGPFDY

SEQ ID NO: 72 - protein, 8 aa, synthetic construct
  REGION 1..8: note = H-CDR3 (SKAI-DS42)
RDGNTFDY

SEQ ID NO: 73 - protein, 8 aa, synthetic construct
  REGION 1..8: note = H-CDR3 (SKAI-DS63)
KYQWDFDY

SEQ ID NO: 74 - protein, 8 aa, synthetic construct
  REGION 1..8: note = H-CDR3 (SKAI-DS64)
RFDPVFDY

SEQ ID NO: 75 - protein, 8 aa, synthetic construct
  REGION 1..8: note = H-CDR3 (SKAI-DS66)
RNLFGFDY

SEQ ID NO: 76 - protein, 8 aa, synthetic construct
  REGION 1..8: note = H-CDR3 (SKAI-DS77)
RSHPTFDY

SEQ ID NO: 77 - protein, 13 aa, synthetic construct
  REGION 1..13: note = H-CDR3 (SKAI-DS84)
RDPFPGRSSNFDY

SEQ ID NO: 78 - protein, 13 aa, synthetic construct
  REGION 1..13: note = H-CDR3 (SKAI-DS95)
KDAWTLHPFSFDY

SEQ ID NO: 79 - protein, 8 aa, synthetic construct
  REGION 1..8: note = H-CDR3 (SKAI-DS104)
KPPTWFDY